European Patent Application EP 4 491 230 A1, published January 15, 2025. Title: ANTIBODIES TARGETING LEUKOCYTE IMMUNOGLOBULIN-LIKE RECEPTOR SUBFAMILY B1 (LILRB1) AND/OR LILRB2, COMBINATIONS AND USES THEREOF. Applicant: iOmx Therapeutics AG. Application EP. The sequence listing filed with the application follows.

SEQUENCE LISTING (395 sequences)

SEQ ID NO: 1 - protein, 5 aa, synthetic construct
SYAIS

SEQ ID NO: 2 - protein, 17 aa, synthetic construct
GIIPIFGTANYAQKFQG

SEQ ID NO: 3 - protein, 17 aa, synthetic construct
DLGTYSSGWPYYYGMDV

SEQ ID NO: 4 - protein, 126 aa, synthetic construct
QVQLVQSGAEVKKPGSSVKVSCKASGGTFSSYAISWVRQAPGQGLEWMGGIIPIFGTANYAQKFQGRVTITADESTSTAYMELSSLRSEDTAVYYCAKDLGTYSSGWPYYYGMDVWGQGTTVTVSS

SEQ ID NO: 5 - protein, 11 aa, synthetic construct
SGDKLGDKYAS

SEQ ID NO: 6 - protein, 7 aa, synthetic construct
QDSKRPS

SEQ ID NO: 7 - protein, 9 aa, synthetic construct
QSTTHTSFV

SEQ ID NO: 8 - protein, 106 aa, synthetic construct
SYELTQPPSVSVSPGQTASITCSGDKLGDKYASWYQQKPGQSPVLVIYQDSKRPSGIPERFSGSNSGNTATLTISGTQAEDEADYYCQSTTHTSFVFGGGTKLTVL

SEQ ID NO: 9 - protein, 5 aa, synthetic construct
SYAIS

SEQ ID NO: 10 - protein, 17 aa, synthetic construct
GIIPIFGTANYAQKFQG

SEQ ID NO: 11 - protein, 14 aa, synthetic construct
VHLYYHFPASYFDY

SEQ ID NO: 12 - protein, 123 aa, synthetic construct
QVQLVQSGAEVKKPGSSVKVSCKASGGTFSSYAISWVRQAPGQGLEWMGGIIPIFGTANYAQKFQGRVTITADESTSTAYMELSSLRSEDTAVYYCARVHLYYHFPASYFDYWGQGTLVTVSS

SEQ ID NO: 13 - protein, 11 aa, synthetic construct
SGDKLGDKYAS

SEQ ID NO: 14 - protein, 7 aa, synthetic construct
QDSKRPS

SEQ ID NO: 15 - protein, 11 aa, synthetic construct
QVTPGLGGVYV

SEQ ID NO: 16 - protein, 108 aa, synthetic construct
SYELTQPPSVSVSPGQTASITCSGDKLGDKYASWYQQKPGQSPVLVIYQDSKRPSGIPERFSGSNSGNTATLTISGTQAEDEADYYCQVTPGLGGVYVFGGGTKLTVL

SEQ ID NO: 17 - protein, 5 aa, synthetic construct
SYAIS

SEQ ID NO: 18 - protein, 17 aa, synthetic construct
GIIPIFGTANYAQKFQG

SEQ ID NO: 19 - protein, 17 aa, synthetic construct
GPPVGSSSWYTDWYFDL

SEQ ID NO: 20 - protein, 126 aa, synthetic construct
QVQLVQSGAEVKKPGSSVKVSCKASGGTFSSYAISWVRQAPGQGLEWMGGIIPIFGTANYAQKFQGRVTITADESTSTAYMELSSLRSEDTAVYYCAKGPPVGSSSWYTDWYFDLWGRGTLVTVSS

SEQ ID NO: 21 - protein, 11 aa, synthetic construct
SGDKLGDKYAS

SEQ ID NO: 22 - protein, 7 aa, synthetic construct
QDSKRPS

SEQ ID NO: 23 - protein, 11 aa, synthetic construct
LSYGAHSHGVV

SEQ ID NO: 24 - protein, 108 aa, synthetic construct
SYELTQPPSVSVSPGQTASITCSGDKLGDKYASWYQQKPGQSPVLVIYQDSKRPSGIPERFSGSNSGNTATLTISGTQAEDEADYYCLSYGAHSHGVVFGGGTKLTVL

SEQ ID NO: 25 - protein, 5 aa, synthetic construct
TKAIA

SEQ ID NO: 26 - protein, 17 aa, synthetic construct
GIIPIFSTANYAPKFQG

SEQ ID NO: 27 - protein, 17 aa, synthetic construct
DLGTYSSGWPYYYGMDV

SEQ ID NO: 28 - protein, 126 aa, synthetic construct
QVQLVQSGAEVKKPGSSVKVSCKASGGTFRTKAIAWVRQAPGQGLEWMGGIIPIFSTANYAPKFQGRVTITADESTSTAYMELSSLRSEDTAVYYCAKDLGTYSSGWPYYYGMDVWGQGTTVTVSS

SEQ ID NO: 29 - protein, 11 aa, synthetic construct
SGDKLGDKYAS

SEQ ID NO: 30 - protein, 7 aa, synthetic construct
QDSKRPS

SEQ ID NO: 31 - protein, 9 aa, synthetic construct
QSTTHTSFV

SEQ ID NO: 32 - protein, 106 aa, synthetic construct; identical to SEQ ID NO: 8

SEQ ID NO: 33 - protein, 5 aa, synthetic construct
IYAIN

SEQ ID NO: 34 - protein, 17 aa, synthetic construct
GIIPGFHSANYAQKFQG

SEQ ID NO: 35 - protein, 17 aa, synthetic construct
DLGTYSSGWPYYYGMDV

SEQ ID NO: 36 - protein, 126 aa, synthetic construct
QVQLVQSGAEVKKPGSSVKVSCKASGGTFTIYAINWVRQAPGQGLEWMGGIIPGFHSANYAQKFQGRVTITADESTSTAYMELSSLRSEDTAVYYCAKDLGTYSSGWPYYYGMDVWGQGTTVTVSS

SEQ ID NO: 37 - protein, 11 aa, synthetic construct
SGDKLGDKYAS

SEQ ID NO: 38 - protein, 7 aa, synthetic construct
QDSKRPS

SEQ ID NO: 39 - protein, 9 aa, synthetic construct
QSTTHTSFV

SEQ ID NO: 40 - protein, 106 aa, synthetic construct; identical to SEQ ID NO: 8

SEQ ID NO: 41 - protein, 5 aa, synthetic construct
QYAFS

SEQ ID NO: 42 - protein, 17 aa, synthetic construct
SIIPGFTTSNYAHKFQG

SEQ ID NO: 43 - protein, 17 aa, synthetic construct
DLGTYSSGWPYYYGMDV

SEQ ID NO: 44 - protein, 126 aa, synthetic construct
QVQLVQSGAEVKKPGSSVKVSCKASGGTFSQYAFSWVRQAPGQGLEWMGSIIPGFTTSNYAHKFQGRVTITADESTSTAYMELSSLRSEDTAVYYCAKDLGTYSSGWPYYYGMDVWGQGTTVTVSS

SEQ ID NO: 45 - protein, 11 aa, synthetic construct
SGDKLGDKYAS

SEQ ID NO: 46 - protein, 7 aa, synthetic construct
QDSKRPS

SEQ ID NO: 47 - protein, 9 aa, synthetic construct
QSTTHTSFV

SEQ ID NO: 48 - protein, 106 aa, synthetic construct; identical to SEQ ID NO: 8

SEQ ID NO: 49 - protein, 5 aa, synthetic construct
EYAFS

SEQ ID NO: 50 - protein, 17 aa, synthetic construct
SIIPTFHTSNYAGKFQG

SEQ ID NO: 51 - protein, 17 aa, synthetic construct
DLGTYSSGWPYYYGMDV

SEQ ID NO: 52 - protein, 126 aa, synthetic construct
QVQLVQSGAEVKKPGSSVKVSCKASGGSFREYAFSWVRQAPGQGLEWMGSIIPTFHTSNYAGKFQGRVTITADESTSTAYMELSSLRSEDTAVYYCAKDLGTYSSGWPYYYGMDVWGQGTTVTVSS

SEQ ID NO: 53 - protein, 11 aa, synthetic construct
SGDKLGDKYAS

SEQ ID NO: 54 - protein, 7 aa, synthetic construct
QDSKRPS

SEQ ID NO: 55 - protein, 9 aa, synthetic construct
QSTTHTSFV

SEQ ID NO: 56 - protein, 106 aa, synthetic construct; identical to SEQ ID NO: 8

SEQ ID NO: 57 - protein, 5 aa, synthetic construct
ESAIL

SEQ ID NO: 58 - protein, 17 aa, synthetic construct
GIVPSFYSANYAQKFQG

SEQ ID NO: 59 - protein, 17 aa, synthetic construct
DLGTYSSGWPYYYGMDV

SEQ ID NO: 60 - protein, 126 aa, synthetic construct
QVQLVQSGAEVKKPGSSVKVSCKASGGTFAESAILWVRQAPGQGLEWMGGIVPSFYSANYAQKFQGRVTITADESTSTAYMELSSLRSEDTAVYYCAKDLGTYSSGWPYYYGMDVWGQGTTVTVSS

SEQ ID NO: 61 - protein, 11 aa, synthetic construct
SGDKLGDKYAS

SEQ ID NO: 62 - protein, 7 aa, synthetic construct
QDSKRPS

SEQ ID NO: 63 - protein, 9 aa, synthetic construct
QSTTHTSFV

SEQ ID NO: 64 - protein, 106 aa, synthetic construct; identical to SEQ ID NO: 8

SEQ ID NO: 65 - protein, 5 aa, synthetic construct
VTAIL

SEQ ID NO: 66 - protein, 17 aa, synthetic construct
GIIPSFTSANYASKFQG

SEQ ID NO: 67 - protein, 17 aa, synthetic construct
DLGTYSSGWPYYYGMDV

SEQ ID NO: 68 - protein, 126 aa, synthetic construct
QVQLVQSGAEVKKPGSSVKVSCKASGGTFSVTAILWVRQAPGQGLEWMGGIIPSFTSANYASKFQGRVTITADESTSTAYMELSSLRSEDTAVYYCAKDLGTYSSGWPYYYGMDVWGQGTTVTVSS

SEQ ID NO: 69 - protein, 11 aa, synthetic construct
SGDKLGDKYAS

SEQ ID NO: 70 - protein, 7 aa, synthetic construct
QDSKRPS

SEQ ID NO: 71 - protein, 9 aa, synthetic construct
QSTTHTSFV

SEQ ID NO: 72 - protein, 106 aa, synthetic construct; identical to SEQ ID NO: 8

SEQ ID NO: 73 - protein, 5 aa, synthetic construct
SQAFA

SEQ ID NO: 74 - protein, 17 aa, synthetic construct
SIIPGFSTANYAQKFQG

SEQ ID NO: 75 - protein, 17 aa, synthetic construct
DLGTYSSGWPYYYGMDV

SEQ ID NO: 76 - protein, 126 aa, synthetic construct
QVQLVQSGAEVKKPGSSVKVSCKASGGTFQSQAFAWVRQAPGQGLEWMGSIIPGFSTANYAQKFQGRVTITADESTSTAYMELSSLRSEDTAVYYCAKDLGTYSSGWPYYYGMDVWGQGTTVTVSS

SEQ ID NO: 77 - protein, 11 aa, synthetic construct
SGDKLGDKYAS

SEQ ID NO: 78 - protein, 7 aa, synthetic construct
QDSKRPS

SEQ ID NO: 79 - protein, 9 aa, synthetic construct
QSTTHTSFV

SEQ ID NO: 80 - protein, 106 aa, synthetic construct; identical to SEQ ID NO: 8

SEQ ID NO: 81 - protein, 5 aa, synthetic construct
HSAFS

SEQ ID NO: 82 - protein, 17 aa, synthetic construct
SIIPAFYTANYAQKFQG

SEQ ID NO: 83 - protein, 17 aa, synthetic construct
DLGTYSSGWPYYYGMDV

SEQ ID NO: 84 - protein, 126 aa, synthetic construct
QVQLVQSGAEVKKPGSSVKVSCKASGGSFSHSAFSWVRQAPGQGLEWMGSIIPAFYTANYAQKFQGRVTITADESTSTAYMELSSLRSEDTAVYYCAKDLGTYSSGWPYYYGMDVWGQGTTVTVSS

SEQ ID NO: 85 - protein, 11 aa, synthetic construct
SGDKLGDKYAS

SEQ ID NO: 86 - protein, 7 aa, synthetic construct
QDSKRPS

SEQ ID NO: 87 - protein, 9 aa, synthetic construct
QSTTHTSFV

SEQ ID NO: 88 - protein, 106 aa, synthetic construct; identical to SEQ ID NO: 8

SEQ ID NO: 89 - protein, 5 aa, synthetic construct
EYAFL

SEQ ID NO: 90 - protein, 17 aa, synthetic construct
GIIPKFHTANYAQKFQG

SEQ ID NO: 91 - protein, 17 aa, synthetic construct
DLGTYSSGWPYYYGMDV

SEQ ID NO: 92 - protein, 126 aa, synthetic construct
QVQLVQSGAEVKKPGSSVKVSCKASGGTISEYAFLWVRQAPGQGLEWMGGIIPKFHTANYAQKFQGRVTITADESTSTAYMELSSLRSEDTAVYYCAKDLGTYSSGWPYYYGMDVWGQGTTVTVSS

SEQ ID NO: 93 - protein, 11 aa, synthetic construct
SGDKLGDKYAS

SEQ ID NO: 94 - protein, 7 aa, synthetic construct
QDSKRPS

SEQ ID NO: 95 - protein, 9 aa, synthetic construct
QSTTHTSFV

SEQ ID NO: 96 - protein, 106 aa, synthetic construct; identical to SEQ ID NO: 8

SEQ ID NO: 97 - protein, 5 aa, synthetic construct
QEAFS

SEQ ID NO: 98 - protein, 17 aa, synthetic construct
SIIPIFYSSNYAQKFQG

SEQ ID NO: 99 - protein, 17 aa, synthetic construct
DLGTYSSGWPYYYGMDV

SEQ ID NO: 100 - protein, 126 aa, synthetic construct
QVQLVQSGAEVKKPGSSVKVSCKASGGTFRQEAFSWVRQAPGQGLEWMGSIIPIFYSSNYAQKFQGRVTITADESTSTAYMELSSLRSEDTAVYYCAKDLGTYSSGWPYYYGMDVWGQGTTVTVSS

SEQ ID NO: 101 - protein, 11 aa, synthetic construct
SGDKLGDKYAS

SEQ ID NO: 102 - protein, 7 aa, synthetic construct
QDSKRPS

SEQ ID NO: 103 - protein, 9 aa, synthetic construct
QSTTHTSFV

SEQ ID NO: 104 - protein, 106 aa, synthetic construct; identical to SEQ ID NO: 8

SEQ ID NO: 105 - protein, 5 aa, synthetic construct
SYAIN

SEQ ID NO: 106 - protein, 17 aa, synthetic construct
GIIPIFHTSNYAQKFQG

SEQ ID NO: 107 - protein, 17 aa, synthetic construct
DLGTYSSGWPYYYGMDV

SEQ ID NO: 108 - protein, 126 aa, synthetic construct
QVQLVQSGAEVKKPGSSVKVSCKASGGTFSSYAINWVRQAPGQGLEWMGGIIPIFHTSNYAQKFQGRVTITADESTSTAYMELSSLRSEDTAVYYCAKDLGTYSSGWPYYYGMDVWGQGTTVTVSS

SEQ ID NO: 109 - protein, 11 aa, synthetic construct
SGDKLGDKYAS

SEQ ID NO: 110 - protein, 7 aa, synthetic construct
QDSKRPS

SEQ ID NO: 111 - protein, 9 aa, synthetic construct
QSTTHTSFV

SEQ ID NO: 112 - protein, 106 aa, synthetic construct; identical to SEQ ID NO: 8

SEQ ID NO: 113 - protein, 5 aa, synthetic construct
SYAIN

SEQ ID NO: 114 - protein, 17 aa, synthetic construct
GIIPGFSTANYAQKFQG

SEQ ID NO: 115 - protein, 17 aa, synthetic construct
DLGTYSSGWPYYYGMDV

SEQ ID NO: 116 - protein, 126 aa, synthetic construct
QVQLVQSGAEVKKPGSSVKVSCKASGGSFQSYAINWVRQAPGQGLEWMGGIIPGFSTANYAQKFQGRVTITADESTSTAYMELSSLRSEDTAVYYCAKDLGTYSSGWPYYYGMDVWGQGTTVTVSS

SEQ ID NO: 117 - protein, 11 aa, synthetic construct
SGDKLGDKYAS

SEQ ID NO: 118 - protein, 7 aa, synthetic construct
QDSKRPS

SEQ ID NO: 119 - protein, 9 aa, synthetic construct
QSTTHTSFV

SEQ ID NO: 120 - protein, 106 aa, synthetic construct; identical to SEQ ID NO: 8

SEQ ID NO: 121 - protein, 5 aa, synthetic construct
SYAFN

SEQ ID NO: 122 - protein, 17 aa, synthetic construct
SIIPIFKTANYAQKFQG

SEQ ID NO: 123 - protein, 17 aa, synthetic construct
DLGTYSSGWPYYYGMDV

SEQ ID NO: 124 - protein, 126 aa, synthetic construct
QVQLVQSGAEVKKPGSSVKVSCKASGGTFSSYAFNWVRQAPGQGLEWMGSIIPIFKTANYAQKFQGRVTITADESTSTAYMELSSLRSEDTAVYYCAKDLGTYSSGWPYYYGMDVWGQGTTVTVSS

SEQ ID NO: 125 - protein, 11 aa, synthetic construct
SGDKLGDKYAS

SEQ ID NO: 126 - protein, 7 aa, synthetic construct
QDSKRPS

SEQ ID NO: 127 - protein, 9 aa, synthetic construct
QSTTHTSFV

SEQ ID NO: 128 - protein, 106 aa, synthetic construct; identical to SEQ ID NO: 8

SEQ ID NO: 129 - protein, 5 aa, synthetic construct
SYAIS

SEQ ID NO: 130 - protein, 17 aa, synthetic construct
GIIPYFSLANYAPKFQG

SEQ ID NO: 131 - protein, 17 aa, synthetic construct
DLGTYSSGWPYYYGMDV

SEQ ID NO: 132 - protein, 126 aa, synthetic construct
QVQLVQSGAEVKKPGSSVKVSCKASGGTFSSYAISWVRQAPGQGLEWMGGIIPYFSLANYAPKFQGRVTITADESTSTAYMELSSLRSEDTAVYYCAKDLGTYSSGWPYYYGMDVWGQGTTVTVSS

SEQ ID NO: 133 - protein, 11 aa, synthetic construct
SGDKLGDKYAS

SEQ ID NO: 134 - protein, 7 aa, synthetic construct
QDSKRPS

SEQ ID NO: 135 - protein, 9 aa, synthetic construct
QSTTHTSFV

SEQ ID NO: 136 - protein, 106 aa, synthetic construct; identical to SEQ ID NO: 8

SEQ ID NO: 137 - protein, 5 aa, synthetic construct
TSAIS

SEQ ID NO: 138 - protein, 17 aa, synthetic construct
GIIPIFYTANYAQKFQG

SEQ ID NO: 139 - protein, 17 aa, synthetic construct
DLGTYSSGWPYYYGMDV

SEQ ID NO: 140 - protein, 126 aa, synthetic construct
QVQLVQSGAEVKKPGSSVKVSCKASGGTFSTSAISWVRQAPGQGLEWMGGIIPIFYTANYAQKFQGRVTITADESTSTAYMELSSLRSEDTAVYYCAKDLGTYSSGWPYYYGMDVWGQGTTVTVSS

SEQ ID NO: 141 - protein, 11 aa, synthetic construct
SGDKLGDKYAS

SEQ ID NO: 142 - protein, 7 aa, synthetic construct
QDSKRPS

SEQ ID NO: 143 - protein, 9 aa, synthetic construct
QSTTHTSFV

SEQ ID NO: 144 - protein, 106 aa, synthetic construct; identical to SEQ ID NO: 8

SEQ ID NO: 145 - protein, 5 aa, synthetic construct
TSAMN

SEQ ID NO: 146 - protein, 17 aa, synthetic construct
GIIPYFSTANYAPKFQG

SEQ ID NO: 147 - protein, 17 aa, synthetic construct
DLGTYSSGWPYYYGMDV

SEQ ID NO: 148 - protein, 126 aa, synthetic construct
QVQLVQSGAEVKKPGSSVKVSCKASGYTFTTSAMNWVRQAPGQGLEWMGGIIPYFSTANYAPKFQGRVTITADESTSTAYMELSSLRSEDTAVYYCAKDLGTYSSGWPYYYGMDVWGQGTTVTVSS

SEQ ID NO: 149 - protein, 11 aa, synthetic construct
SGDKLGDKYAS

SEQ ID NO: 150 - protein, 7 aa, synthetic construct
QDSKRPS

SEQ ID NO: 151 - protein, 9 aa, synthetic construct
QSTTHTSFV

SEQ ID NO: 152 - protein, 106 aa, synthetic construct; identical to SEQ ID NO: 8

SEQ ID NO: 153 - protein, 5 aa, synthetic construct
TYAIS

SEQ ID NO: 154 - protein, 17 aa, synthetic construct
SIIPKFYQSNYAYKFQG

SEQ ID NO: 155 - protein, 17 aa, synthetic construct
DLGTYSSGWPYYYGMDV

SEQ ID NO: 156 - protein, 126 aa, synthetic construct
QVQLVQSGAEVKKPGSSVKVSCKASGGTFQTYAISWVRQAPGQGLEWMGSIIPKFYQSNYAYKFQGRVTITADESTSTAYMELSSLRSEDTAVYYCAKDLGTYSSGWPYYYGMDVWGQGTTVTVSS

SEQ ID NO: 157 - protein, 11 aa, synthetic construct
SGDKLGDKYAS

SEQ ID NO: 158 - protein, 7 aa, synthetic construct
QDSKRPS

SEQ ID NO: 159 - protein, 9 aa, synthetic construct
QSTTHTSFV

SEQ ID NO: 160 - protein, 106 aa, synthetic construct; identical to SEQ ID NO: 8

SEQ ID NO: 161 - protein, 5 aa, synthetic construct
SYAFA

SEQ ID NO: 162 - protein, 17 aa, synthetic construct
GIIPGFYAANYAQKFQG

SEQ ID NO: 163 - protein, 17 aa, synthetic construct
DLGTYSSGWPYYYGMDV

SEQ ID NO: 164 - protein, 126 aa, synthetic construct
QVQLVQSGAEVKKPGSSVKVSCKASGGSITSYAFAWVRQAPGQGLEWMGGIIPGFYAANYAQKFQGRVTITADESTSTAYMELSSLRSEDTAVYYCAKDLGTYSSGWPYYYGMDVWGQGTTVTVSS

SEQ ID NO: 165 - protein, 11 aa, synthetic construct
SGDKLGDKYAS

SEQ ID NO: 166 - protein, 7 aa, synthetic construct
QDSKRPS

SEQ ID NO: 167 - protein, 9 aa, synthetic construct
QSTTHTSFV

SEQ ID NO: 168 - protein, 106 aa, synthetic construct; identical to SEQ ID NO: 8

SEQ ID NO: 169 - protein, 5 aa, synthetic construct
GSAIS

SEQ ID NO: 170 - protein, 17 aa, synthetic construct
GIVLAYSTSVYAQKFQG

SEQ ID NO: 171 - protein, 17 aa, synthetic construct
GPPVGSSSWYTDWYFDL

SEQ ID NO: 172 - protein, 126 aa, synthetic construct
QVQLVQSGAEVKKPGSSVKVSCKASGGTFGGSAISWVRQAPGQGLEWMGGIVLAYSTSVYAQKFQGRVTITADESTSTAYMELSSLRSEDTAVYYCAKGPPVGSSSWYTDWYFDLWGRGTLVTVSS

SEQ ID NO: 173 - protein, 11 aa, synthetic construct
SGDKLGDKYAS

SEQ ID NO: 174 - protein, 7 aa, synthetic construct
QDSKRPS

SEQ ID NO: 175 - protein, 11 aa, synthetic construct
LSYGAHSHGVV

SEQ ID NO: 176 - protein, 108 aa, synthetic construct; identical to SEQ ID NO: 24

SEQ ID NO: 177 - protein, 5 aa, synthetic construct
QYAMS

SEQ ID NO: 178 - protein, 17 aa, synthetic construct
GIIPQFSTSVYAQKFQG

SEQ ID NO: 179 - protein, 17 aa, synthetic construct
GPPVGSSSWYTDWYFDL

SEQ ID NO: 180 - protein, 126 aa, synthetic construct
QVQLVQSGAEVKKPGSSVKVSCKASGYTFQQYAMSWVRQAPGQGLEWIGGIIPQFSTSVYAQKFQGRVTITADESTSTAYMELSSLRSEDTAVYYCAKGPPVGSSSWYTDWYFDLWGRGTLVTVSS

SEQ ID NO: 181 - protein, 11 aa, synthetic construct
SGDKLGDKYAS

SEQ ID NO: 182 - protein, 7 aa, synthetic construct
QDSKRPS

SEQ ID NO: 183 - protein, 11 aa, synthetic construct
LSYGAHSHGVV

SEQ ID NO: 184 - protein, 108 aa, synthetic construct; identical to SEQ ID NO: 24

SEQ ID NO: 185 - protein, 5 aa, synthetic construct
GSAMS

SEQ ID NO: 186 - protein, 17 aa, synthetic construct
GILPIFGTSVYAQKFQG

SEQ ID NO: 187 - protein, 17 aa, synthetic construct
GPPVGSSSWYTDWYFDL

SEQ ID NO: 188 - protein, 126 aa, synthetic construct
QVQLVQSGAEVKKPGSSVKVSCKASGYTFTGSAMSWVRQAPGQGLEWMGGILPIFGTSVYAQKFQGRVTITADESTSTAYMELSSLRSEDTAVYYCAKGPPVGSSSWYTDWYFDLWGRGTLVTVSS

SEQ ID NO: 189 - protein, 11 aa, synthetic construct
SGDKLGDKYAS

SEQ ID NO: 190 - protein, 7 aa, synthetic construct
QDSKRPS

SEQ ID NO: 191 - protein, 11 aa, synthetic construct
LSYGAHSHGVV

SEQ ID NO: 192 - protein, 108 aa, synthetic construct; identical to SEQ ID NO: 24

SEQ ID NO: 193 - protein, 5 aa, synthetic construct
KSAMS

SEQ ID NO: 194 - protein, 17 aa, synthetic construct
GIVPKFHTSVYAQKFQG

SEQ ID NO: 195 - protein, 17 aa, synthetic construct
GPPVGSSSWYTDWYFDL

SEQ ID NO: 196 - protein, 126 aa, synthetic construct
QVQLVQSGAEVKKPGSSVKVSCKASGYTFSKSAMSWVRQAPGQGLEWMGGIVPKFHTSVYAQKFQGRVTITADESTSTAYMELSSLRSEDTAVYYCAKGPPVGSSSWYTDWYFDLWGRGTLVTVSS

SEQ ID NO: 197 - protein, 11 aa, synthetic construct
SGDKLGDKYAS

SEQ ID NO: 198 - protein, 7 aa, synthetic construct
QDSKRPS

SEQ ID NO: 199 - protein, 11 aa, synthetic construct
LSYGAHSHGVV

SEQ ID NO: 200 - protein, 108 aa, synthetic construct; identical to SEQ ID NO: 24

SEQ ID NO: 201 - protein, 5 aa, synthetic construct
SHGMS

SEQ ID NO: 202 - protein, 17 aa, synthetic construct
GILPIFHTATYAQKFQG

SEQ ID NO: 203 - protein, 17 aa, synthetic construct
GPPVGSSSWYTDWYFDL

SEQ ID NO: 204 - protein, 126 aa, synthetic construct
QVQLVQSGAEVKKPGSSVKVSCKASGYTFTSHGMSWVRQAPGQGLEWMGGILPIFHTATYAQKFQGRVTITADESTSTAYMELSSLRSEDTAVYYCAKGPPVGSSSWYTDWYFDLWGRGTLVTVSS

SEQ ID NO: 205 - protein, 11 aa, synthetic construct
SGDKLGDKYAS

SEQ ID NO: 206 - protein, 7 aa, synthetic construct
QDSKRPS

SEQ ID NO: 207 - protein, 11 aa, synthetic construct
LSYGAHSHGVV

SEQ ID NO: 208 - protein, 108 aa, synthetic construct; identical to SEQ ID NO: 24

SEQ ID NO: 209 - protein, 5 aa, synthetic construct
GYAIS

SEQ ID NO: 210 - protein, 17 aa, synthetic construct
GILPSFYTAVYAQKFQG

SEQ ID NO: 211 - protein, 17 aa, synthetic construct
GPPVGSSSWYTDWYFDL

SEQ ID NO: 212 - protein, 126 aa, synthetic construct
QVQLVQSGAEVKKPGSSVKVSCKASGGSFTGYAISWVRQAPGQGLEWMGGILPSFYTAVYAQKFQGRVTITADESTSTAYMELSSLRSEDTAVYYCAKGPPVGSSSWYTDWYFDLWGRGTLVTVSS

SEQ ID NO: 213 - protein, 11 aa, synthetic construct
SGDKLGDKYAS

SEQ ID NO: 214 - protein, 7 aa, synthetic construct
QDSKRPS

SEQ ID NO: 215 - protein, 11 aa, synthetic construct
LSYGAHSHGVV

SEQ ID NO: 216 - protein, 108 aa, synthetic construct; identical to SEQ ID NO: 24

SEQ ID NO: 217 - protein, 5 aa, synthetic construct
EHAMS

SEQ ID NO: 218 - protein, 17 aa, synthetic construct
GIIPKFSTSVFAQKFQG

SEQ ID NO: 219 - protein, 17 aa, synthetic construct
GPPVGSSSWYTDWYFDL

SEQ ID NO: 220 - protein, 126 aa, synthetic construct
QVQLVQSGAEVKKPGSSVKVSCKASGYSFSEHAMSWVRQAPGQGLEWMGGIIPKFSTSVFAQKFQGRVTITADESTSTAYMELSSLRSEDTAVYYCAKGPPVGSSSWYTDWYFDLWGRGTLVTVSS

SEQ ID NO: 221 - protein, 11 aa, synthetic construct
SGDKLGDKYAS

SEQ ID NO: 222 - protein, 7 aa, synthetic construct
QDSKRPS

SEQ ID NO: 223 - protein, 11 aa, synthetic construct
LSYGAHSHGVV

SEQ ID NO: 224 - protein, 108 aa, synthetic construct; identical to SEQ ID NO: 24

SEQ ID NO: 225 - protein, 5 aa, synthetic construct
IYAMS

SEQ ID NO: 226 - protein, 17 aa, synthetic construct
GIIPSFRTAVYAQKFQG

SEQ ID NO: 227 - protein, 17 aa, synthetic construct
GPPVGSSSWYTDWYFDL

SEQ ID NO: 228 - protein, 126 aa, synthetic construct
QVQLVQSGAEVKKPGSSVKVSCKASGYTFSIYAMSWVRQAPGQGLEWMGGIIPSFRTAVYAQKFQGRVTITADESTSTAYMELSSLRSEDTAVYYCAKGPPVGSSSWYTDWYFDLWGRGTLVTVSS

SEQ ID NO: 229 - protein, 11 aa, synthetic construct
SGDKLGDKYAS

SEQ ID NO: 230 - protein, 7 aa, synthetic construct
QDSKRPS

SEQ ID NO: 231 - protein, 11 aa, synthetic construct
LSYGAHSHGVV

SEQ ID NO: 232 - protein, 108 aa, synthetic construct; identical to SEQ ID NO: 24

SEQ ID NO: 233 - protein, 5 aa, synthetic construct
SYAFS

SEQ ID NO: 234 - protein, 17 aa, synthetic construct
GIVPIYYTATYAQKFQG

SEQ ID NO: 235 - protein, 17 aa, synthetic construct
GPPVGSSSWYTDWYFDL

SEQ ID NO: 236 - protein, 126 aa, synthetic construct
QVQLVQSGAEVKKPGSSVKVSCKASGGSFQSYAFSWVRQAPGQGLEWMGGIVPIYYTATYAQKFQGRVTITADESTSTAYMELSSLRSEDTAVYYCAKGPPVGSSSWYTDWYFDLWGRGTLVTVSS

SEQ ID NO: 237 - protein, 11 aa, synthetic construct
SGDKLGDKYAS

SEQ ID NO: 238 - protein, 7 aa, synthetic construct
QDSKRPS

SEQ ID NO: 239 - protein, 11 aa, synthetic construct
LSYGAHSHGVV

SEQ ID NO: 240 - protein, 108 aa, synthetic construct; identical to SEQ ID NO: 24

SEQ ID NO: 241 - protein, 5 aa, synthetic construct
KTAMS

SEQ ID NO: 242 - protein, 17 aa, synthetic construct
GIIPSYYTAVYAQKFQG

SEQ ID NO: 243 - protein, 17 aa, synthetic construct
GPPVGSSSWYTDWYFDL

SEQ ID NO: 244 - protein, 126 aa, synthetic construct
QVQLVQSGAEVKKPGSSVKVSCKASGYTFTKTAMSWVRQAPGQGLEWMGGIIPSYYTAVYAQKFQGRVTITADESTSTAYMELSSLRSEDTAVYYCAKGPPVGSSSWYTDWYFDLWGRGTLVTVSS

SEQ ID NO: 245 - protein, 11 aa, synthetic construct
SGDKLGDKYAS

SEQ ID NO: 246 - protein, 7 aa, synthetic construct
QDSKRPS

SEQ ID NO: 247 - protein, 11 aa, synthetic construct
LSYGAHSHGVV

SEQ ID NO: 248 - protein, 108 aa, synthetic construct; identical to SEQ ID NO: 24

SEQ ID NO: 249 - protein, 5 aa, synthetic construct
SYAFS

SEQ ID NO: 250 - protein, 17 aa, synthetic construct
GIVPQYSTAVYAQKFQG

SEQ ID NO: 251 - protein, 17 aa, synthetic construct
GPPVGSSSWYTDWYFDL

SEQ ID NO: 252 - protein, 126 aa, synthetic construct
QVQLVQSGAEVKKPGSSVKVSCKASGGTFQSYAFSWVRQAPGQGLEWMGGIVPQYSTAVYAQKFQGRVTITADESTSTAYMELSSLRSEDTAVYYCAKGPPVGSSSWYTDWYFDLWGRGTLVTVSS

SEQ ID NO: 253 - protein, 11 aa, synthetic construct
SGDKLGDKYAS

SEQ ID NO: 254 - protein, 7 aa, synthetic construct
QDSKRPS

SEQ ID NO: 255 - protein, 11 aa, synthetic construct
LSYGAHSHGVV

SEQ ID NO: 256 - protein, 108 aa, synthetic construct; identical to SEQ ID NO: 24

SEQ ID NO: 257 - protein, 5 aa, synthetic construct
SHAMS

SEQ ID NO: 258 - protein, 17 aa, synthetic construct
GIIPTFKTAVFAQKFQG

SEQ ID NO: 259 - protein, 17 aa, synthetic construct
GPPVGSSSWYTDWYFDL

SEQ ID NO: 260 - protein, 126 aa, synthetic construct
QVQLVQSGAEVKKPGSSVKVSCKASGYTFSSHAMSWVRQAPGQGLEWMGGIIPTFKTAVFAQKFQGRVTITADESTSTAYMELSSLRSEDTAVYYCAKGPPVGSSSWYTDWYFDLWGRGTLVTVSS

SEQ ID NO: 261 - protein, 11 aa, synthetic construct
SGDKLGDKYAS

SEQ ID NO: 262 - protein, 7 aa, synthetic construct
QDSKRPS

SEQ ID NO: 263 - protein, 11 aa, synthetic construct
LSYGAHSHGVV

SEQ ID NO: 264 - protein, 108 aa, synthetic construct; identical to SEQ ID NO: 24

SEQ ID NO: 265 - protein, 5 aa, synthetic construct
SYAIS

SEQ ID NO: 266 - protein, 17 aa, synthetic construct
GIIPIFGTANYAQKFQG

SEQ ID NO: 267 - protein, 17 aa, synthetic construct
DLGTYSSGWPYYYGMDV

SEQ ID NO: 268 - protein, 126 aa, synthetic construct; identical to SEQ ID NO: 4

SEQ ID NO: 269 - protein, 11 aa, synthetic construct
SGDKLGDKYAS

SEQ ID NO: 270 - protein, 7 aa, synthetic construct
QDSKRPS

SEQ ID NO: 271 - protein, 9 aa, synthetic construct
QLYGHTITV

SEQ ID NO: 272 - protein, 106 aa, synthetic construct
SYELTQPPSVSVSPGQTASITCSGDKLGDKYASWYQQKPGQSPVLVIYQDSKRPSGIPERFSGSNSGNTATLTISGTQAEDEADYYCQLYGHTITVFGGGTKLTVL

SEQ ID NO: 273 - protein, 5 aa, synthetic construct
SYAIS

SEQ ID NO: 274 - protein, 17 aa, synthetic construct
GIIPIFGTANYAQKFQG

SEQ ID NO: 275 - protein, 17 aa, synthetic construct
DLGTYSSGWPYYYGMDV

SEQ ID NO: 276 - protein, 126 aa, synthetic construct; identical to SEQ ID NO: 4

SEQ ID NO: 277 - protein, 11 aa, synthetic construct
SGDKLGDKYAS

SEQ ID NO: 278 - protein, 7 aa, synthetic construct
QDSKRPS

SEQ ID NO: 279 - protein, 9 aa, synthetic construct
QLSHGTLLV

SEQ ID NO: 280 - protein, 106 aa, synthetic construct
SYELTQPPSVSVSPGQTASITCSGDKLGDKYASWYQQKPGQSPVLVIYQDSKRPSGIPERFSGSNSGNTATLTISGTQAEDEADYYCQLSHGTLLVFGGGTKLTVL

SEQ ID NO: 281 - protein, 5 aa, synthetic construct
SYAIS

SEQ ID NO: 282 - protein, 17 aa, synthetic construct
GIIPIFGTANYAQKFQG

SEQ ID NO: 283 - protein, 17 aa, synthetic construct
DLGTYSSGWPYYYGMDV

SEQ ID NO: 284 - protein, 126 aa, synthetic construct; identical to SEQ ID NO: 4

SEQ ID NO: 285 - protein, 11 aa, synthetic construct
SGDKLGDKYAS

SEQ ID NO: 286 - protein, 7 aa, synthetic construct
QDSKRPS

SEQ ID NO: 287 - protein, 9 aa, synthetic construct
QLTHLTIYV

SEQ ID NO: 288 - protein, 106 aa, synthetic construct
SYELTQPPSVSVSPGQTASITCSGDKLGDKYASWYQQKPGQSPVLVIYQDSKRPSGIPERFSGSNSGNTATLTISGTQAEDEADYYCQLTHLTIYVFGGGTKLTVL

SEQ ID NO: 289 - protein, 5 aa, synthetic construct
SYAIS

SEQ ID NO: 290 - protein, 17 aa, synthetic construct
GIIPIFGTANYAQKFQG

SEQ ID NO: 291 - protein, 14 aa, synthetic construct
VHLYYHFPASYFDY

SEQ ID NO: 292 - protein, 123 aa, synthetic construct; identical to SEQ ID NO: 12

SEQ ID NO: 293 - protein, 11 aa, synthetic construct
SGDKLGDKYAS

SEQ ID NO: 294 - protein, 7 aa, synthetic construct
QDSKRPS

SEQ ID NO: 295 - protein, 11 aa, synthetic construct
LASLGTGGVYV

SEQ ID NO: 296 - protein, 108 aa, synthetic construct
SYELTQPPSVSVSPGQTASITCSGDKLGDKYASWYQQKPGQSPVLVIYQDSKRPSGIPERFSGSNSGNTATLTISGTQAEDEADYYCLASLGTGGVYVFGGGTKLTVL

SEQ ID NO: 297 - protein, 5 aa, synthetic construct
SYAIS

SEQ ID NO: 298 - protein, 17 aa, synthetic construct
GIIPIFGTANYAQKFQG

SEQ ID NO: 299 - protein, 17 aa, synthetic construct
GPPVGSSSWYTDWYFDL

SEQ ID NO: 300 - protein, 126 aa, synthetic construct; identical to SEQ ID NO: 20

SEQ ID NO: 301 - protein, 11 aa, synthetic construct
SGDKLGDKYAS

SEQ ID NO: 302 - protein, 7 aa, synthetic construct
QDSKRPS

SEQ ID NO: 303 - protein, 10 aa, synthetic construct
SLYGAGHTVV

SEQ ID NO: 304 - protein, 107 aa, synthetic construct
SYELTQPPSVSVSPGQTASITCSGDKLGDKYASWYQQKPGQSPVLVIYQDSKRPSGIPERFSGSNSGNTATLTISGTQAEDEADYYCSLYGAGHTVVFGGGTKLTVL

SEQ ID NO: 305 - protein, 5 aa, synthetic construct
SYAIS

SEQ ID NO: 306 - protein, 17 aa, synthetic construct
GIIPIFGTANYAQKFQG

SEQ ID NO: 307 - protein, 17 aa, synthetic construct
GPPVGSSSWYTDWYFDL

SEQ ID NO: 308 - protein, 126 aa, synthetic construct; identical to SEQ ID NO: 20

SEQ ID NO: 309 - protein, 11 aa, synthetic construct
SGDKLGDKYAS

SEQ ID NO: 310 - protein, 7 aa, synthetic construct
QDSKRPS

SEQ ID NO: 311 - protein, 10 aa, synthetic construct
ALYGGGHTVV

SEQ ID NO: 312 - protein, 107 aa, synthetic construct
SYELTQPPSVSVSPGQTASITCSGDKLGDKYASWYQQKPGQSPVLVIYQDSKRPSGIPERFSGSNSGNTATLTISGTQAEDEADYYCALYGGGHTVVFGGGTKLTVL

SEQ ID NO: 313 - protein, 5 aa, synthetic construct
SYAIS

SEQ ID NO: 314 - protein, 17 aa, synthetic construct
GIIPIFGTANYAQKFQG

SEQ ID NO: 315 - protein, 17 aa, synthetic construct
GPPVGSSSWYTDWYFDL

SEQ ID NO: 316 - protein, 126 aa, synthetic construct; identical to SEQ ID NO: 20

SEQ ID NO: 317 - protein, 11 aa, synthetic construct
SGDKLGDKYAS

SEQ ID NO: 318 - protein, 7 aa, synthetic construct
QDSKRPS

SEQ ID NO: 319 - protein, 10 aa, synthetic construct
SLYGPAHTGV

SEQ ID NO: 320 - protein, 107 aa, synthetic construct
SYELTQPPSVSVSPGQTASITCSGDKLGDKYASWYQQKPGQSPVLVIYQDSKRPSGIPERFSGSNSGNTATLTISGTQAEDEADYYCSLYGPAHTGVFGGGTKLTVL

SEQ ID NO: 321 - protein, 5 aa, synthetic construct
SYAIS

SEQ ID NO: 322 - protein, 17 aa, synthetic construct
GIIPIFGTANYAQKFQG

SEQ ID NO: 323 - protein, 17 aa, synthetic construct
GPPVGSSSWYTDWYFDL

SEQ ID NO: 324 - protein, 126 aa, synthetic construct; identical to SEQ ID NO: 20

SEQ ID NO: 325 - protein, 11 aa, synthetic construct
SGDKLGDKYAS

SEQ ID NO: 326 - protein, 7 aa, synthetic construct
QDSKRPS

SEQ ID NO: 327 - protein, 10 aa, synthetic construct
SSYGSGLTVV

SEQ ID NO: 328 - protein, 107 aa, synthetic construct
SYELTQPPSVSVSPGQTASITCSGDKLGDKYASWYQQKPGQSPVLVIYQDSKRPSGIPERFSGSNSGNTATLTISGTQAEDEADYYCSSYGSGLTVVFGGGTKLTVL

SEQ ID NO: 329 - protein, 5 aa, synthetic construct
SYAIS

SEQ ID NO: 330 - protein, 17 aa, synthetic construct
GIIPIFGTANYAQKFQG

SEQ ID NO: 331 - protein, 17 aa, synthetic construct
GPPVGSSSWYTDWYFDL

SEQ ID NO: 332 - protein, 126 aa, synthetic construct; identical to SEQ ID NO: 20

SEQ ID NO: 333 - protein, 11 aa, synthetic construct
SGDKLGDKYAS

SEQ ID NO: 334 - protein, 7 aa, synthetic construct
QDSKRPS

SEQ ID NO: 335 - protein, 10 aa, synthetic construct
GVYSSGLTVV

SEQ ID NO: 336 - protein, 107 aa, synthetic construct
SYELTQPPSVSVSPGQTASITCSGDKLGDKYASWYQQKPGQSPVLVIYQDSKRPSGIPERFSGSNSGNTATLTISGTQAEDEADYYCGVYSSGLTVVFGGGTKLTVL

SEQ ID NO: 337 - protein, 5 aa, synthetic construct
SYAIS

SEQ ID NO: 338 - protein, 17 aa, synthetic construct
GIIPIFGTANYAQKFQG

SEQ ID NO: 339 - protein, 17 aa, synthetic construct
GPPVGSSSWYTDWYFDL

SEQ ID NO: 340 - protein, 126 aa, synthetic construct; identical to SEQ ID NO: 20

SEQ ID NO: 341 - protein, 11 aa, synthetic construct
SGDKLGDKYAS

SEQ ID NO: 342 - protein, 7 aa, synthetic construct
QDSKRPS

SEQ ID NO: 343 - protein, 10 aa, synthetic construct
SAYGSGLAVV

SEQ ID NO: 344 - protein, 107 aa, synthetic construct
SYELTQPPSVSVSPGQTASITCSGDKLGDKYASWYQQKPGQSPVLVIYQDSKRPSGIPERFSGSNSGNTATLTISGTQAEDEADYYCSAYGSGLAVVFGGGTKLTVL

SEQ ID NO: 345 - protein, 5 aa, synthetic construct
SYAIS

SEQ ID NO: 346 - protein, 17 aa, synthetic construct
GIIPIFGTANYAQKFQG

SEQ ID NO: 347 - protein, 17 aa, synthetic construct
GPPVGSSSWYTDWYFDL

SEQ ID NO: 348 - protein, 126 aa, synthetic construct; identical to SEQ ID NO: 20

SEQ ID NO: 349 - protein, 11 aa, synthetic construct
SGDKLGDKYAS

SEQ ID NO: 350 - protein, 7 aa, synthetic construct
QDSKRPS

SEQ ID NO: 351 - protein, 10 aa, synthetic construct
SLYASGLIAV

SEQ ID NO: 352 - protein, 107 aa, synthetic construct
SYELTQPPSVSVSPGQTASITCSGDKLGDKYASWYQQKPGQSPVLVIYQDSKRPSGIPERFSGSNSGNTATLTISGTQAEDEADYYCSLYASGLIAVFGGGTKLTVL

SEQ ID NO: 353 - protein, 5 aa, synthetic construct
SQAFA

SEQ ID NO: 354 - protein, 17 aa, synthetic construct
SIIPGFSTANYAQKFQG

SEQ ID NO: 355 - protein, 17 aa, synthetic construct
DLGTYSSGWPYYYGMDV

SEQ ID NO: 356 - protein, 126 aa, synthetic construct; identical to SEQ ID NO: 76

SEQ ID NO: 357 - protein, 11 aa, synthetic construct
SGDKLGDKYAS

SEQ ID NO: 358 - protein, 7 aa, synthetic construct
QDSKRPS

SEQ ID NO: 359 - protein, 9 aa, synthetic construct
QLTHLTIYV

SEQ ID NO: 360 - protein, 106 aa, synthetic construct; identical to SEQ ID NO: 288

SEQ ID NO: 361 - protein, 5 aa, synthetic construct
SYAIN

SEQ ID NO: 362 - protein, 17 aa, synthetic construct
GIIPGFSTANYAQKFQG

SEQ ID NO: 363 - protein, 17 aa, synthetic construct
DLGTYSSGWPYYYGMDV

SEQ ID NO: 364 - protein, 126 aa, synthetic construct; identical to SEQ ID NO: 116

SEQ ID NO: 365 - protein, 11 aa, synthetic construct
SGDKLGDKYAS

SEQ ID NO: 366 - protein, 7 aa, synthetic construct
QDSKRPS

SEQ ID NO: 367 - protein, 9 aa, synthetic construct
QLTHLTIYV

SEQ ID NO: 368 - protein, 106 aa, synthetic construct; identical to SEQ ID NO: 288

SEQ ID NO: 369 - protein, 5 aa, synthetic construct
KSAMS

SEQ ID NO: 370 - protein, 17 aa, synthetic construct
GIVPKFHTSVYAQKFQG

SEQ ID NO: 371 - protein, 17 aa, synthetic construct
GPPVGSSSWYTDWYFDL

SEQ ID NO: 372 - protein, 126 aa, synthetic construct; identical to SEQ ID NO: 196

SEQ ID NO: 373 - protein, 11 aa, synthetic construct
SGDKLGDKYAS

SEQ ID NO: 374 - protein, 7 aa, synthetic construct
QDSKRPS

SEQ ID NO: 375 - protein, 10 aa, synthetic construct
SLYGAGHTVV

SEQ ID NO: 376 - protein, 107 aa, synthetic construct; identical to SEQ ID NO: 304

SEQ ID NO: 377 - protein, 5 aa, synthetic construct
KSAMS

SEQ ID NO: 378 - protein, 17 aa, synthetic construct
GIVPKFHTSVYAQKFQG

SEQ ID NO: 379 - protein, 17 aa, synthetic construct
GPPVGSSSWYTDWYFDL

SEQ ID NO: 380 - protein, 126 aa, synthetic construct; identical to SEQ ID NO: 196

SEQ ID NO: 381 - protein, 11 aa, synthetic construct
SGDKLGDKYAS

SEQ ID NO: 382 - protein, 7 aa, synthetic construct
QDSKRPS

SEQ ID NO: 383 - protein, 10 aa, synthetic construct
ALYGGGHTVV

SEQ ID NO: 384 - protein, 107 aa, synthetic construct; identical to SEQ ID NO: 312

SEQ ID NO: 385 - protein, 650 aa, Homo sapiens
MTPILTVLICLGLSLGPRTHVQAGHLPKPTLWAEPGSVITQGSPVTLRCQGGQETQEYRLYREKKTALWITRIPQELVKKGQFPIPSITWEHAGRYRCYYGSDTAGRSESSDPLELVVTGAYIKPTLSAQPSPVVNSGGNVILQCDSQVAFDGFSLCKEGEDEHPQCLNSQPHARGSSRAIFSVGPVSPSRRWWYRCYAYDSNSPYEWSLPSDLLELLVLGVSKKPSLSVQPGPIVAPEETLTLQCGSDAGYNRFVLYKDGERDFLQLAGAQPQAGLSQANFTLGPVSRSYGGQYRCYGAHNLSSEWSAPSDPLDILIAGQFYDRVSLSVQPGPTVASGENVTLLCQSQGWMQTFLLTKEGAADDPWRLRSTYQSQKYQAEFPMGPVTSAHAGTYRCYGSQSSKPYLLTHPSDPLELVVSGPSGGPSSPTTGPTSTSGPEDQPLTPTGSDPQSGLGRHLGVVIGILVAVILLLLLLLLLFLILRHRRQGKHWTSTQRKADFQHPAGAVGPEPTDRGLQWRSSPAADAQEENLYAAVKHTQPEDGVEMDTRSPHDEDPQAVTYAEVKHSRPRREMASPPSPLSGEFLDTKDRQAEEDRQMDTEAAASEAPQDVTYAQLHSLTLRREATEPPPSQEGPSPAVPSIYATLAIH

SEQ ID NO: 386 - protein, 651 aa, Homo sapiens
MTPILTVLICLGLSLGPRTHVQAGHLPKPTLWAEPGSVITQGSPVTLRCQGGQETQEYRLYREKKTALWITRIPQELVKKGQFPIPSITWEHAGRYRCYYGSDTAGRSESSDPLELVVTGAYIKPTLSAQPSPVVNSGGNVILQCDSQVAFDGFSLCKEGEDEHPQCLNSQPHARGSSRAIFSVGPVSPSRRWWYRCYAYDSNSPYEWSLPSDLLELLVLGVSKKPSLSVQPGPIVAPEETLTLQCGSDAGYNRFVLYKDGERDFLQLAGAQPQAGLSQANFTLGPVSRSYGGQYRCYGAHNLSSEWSAPSDPLDILIAGQFYDRVSLSVQPGPTVASGENVTLLCQSQGWMQTFLLTKEGAADDPWRLRSTYQSQKYQAEFPMGPVTSAHAGTYRCYGSQSSKPYLLTHPSDPLELVVSGPSGGPSSPTTGPTSTSAGPEDQPLTPTGSDPQSGLGRHLGVVIGILVAVILLLLLLLLLFLILRHRRQGKHWTSTQRKADFQHPAGAVGPEPTDRGLQWRSSPAADAQEENLYAAVKHTQPEDGVEMDTRSPHDEDPQAVTYAEVKHSRPRREMASPPSPLSGEFLDTKDRQAEEDRQMDTEAAASEAPQDVTYAQLHSLTLRREATEPPPSQEGPSPAVPSIYATLAIH

SEQ ID NO: 387 - protein, 652 aa, Homo sapiens
MTPILTVLICLGLSLGPRTHVQAGHLPKPTLWAEPGSVITQGSPVTLRCQGGQETQEYRLYREKKTALWITRIPQELVKKGQFPIPSITWEHAGRYRCYYGSDTAGRSESSDPLELVVTGAYIKPTLSAQPSPVVNSGGNVILQCDSQVAFDGFSLCKEGEDEHPQCLNSQPHARGSSRAIFSVGPVSPSRRWWYRCYAYDSNSPYEWSLPSDLLELLVLGVSKKPSLSVQPGPIVAPEETLTLQCGSDAGYNRFVLYKDGERDFLQLAGAQPQAGLSQANFTLGPVSRSYGGQYRCYGAHNLSSEWSAPSDPLDILIAGQFYDRVSLSVQPGPTVASGENVTLLCQSQGWMQTFLLTKEGAADDPWRLRSTYQSQKYQAEFPMGPVTSAHAGTYRCYGSQSSKPYLLTHPSDPLELVVSGPSGGPSSPTTGPTSTSAGPEDQPLTPTGSDPQSGLGRHLGVVIGILVAVILLLLLLLLLFLILRHRRQGKHWTSTQRKADFQHPAGAVGPEPTDRGLQWRSSPAADAQEENLYAAVKHTQPEDGVEMDTRQSPHDEDPQAVTYAEVKHSRPRREMASPPSPLSGEFLDTKDRQAEEDRQMDTEAAASEAPQDVTYAQLHSLTLRREATEPPPSQEGPSPAVPSIYATLAIH

SEQ ID NO: 388 - protein, 651 aa, Homo sapiens
MTPILTVLICLGLSLGPRTHVQAGHLPKPTLWAEPGSVITQGSPVTLRCQGGQETQEYRLYREKKTALWITRIPQELVKKGQFPIPSITWEHAGRYRCYYGSDTAGRSESSDPLELVVTGAYIKPTLSAQPSPVVNSGGNVILQCDSQVAFDGFSLCKEGEDEHPQCLNSQPHARGSSRAIFSVGPVSPSRRWWYRCYAYDSNSPYEWSLPSDLLELLVLGVSKKPSLSVQPGPIVAPEETLTLQCGSDAGYNRFVLYKDGERDFLQLAGAQPQAGLSQANFTLGPVSRSYGGQYRCYGAHNLSSEWSAPSDPLDILIAGQFYDRVSLSVQPGPTVASGENVTLLCQSQGWMQTFLLTKEGAADDPWRLRSTYQSQKYQAEFPMGPVTSAHAGTYRCYGSQSSKPYLLTHPSDPLELVVSGPSGGPSSPTTGPTSTSGPEDQPLTPTGSDPQSGLGRHLGVVIGILVAVILLLLLLLLLFLILRHRRQGKHWTSTQRKADFQHPAGAVGPEPTDRGLQWRSSPAADAQEENLYAAVKHTQPEDGVEMDTRQSPHDEDPQAVTYAEVKHSRPRREMASPPSPLSGEFLDTKDRQAEEDRQMDTEAAASEAPQDVTYAQLHSLTLRREATEPPPSQEGPSPAVPSIYATLAIH

SEQ ID NO: 389 - protein, 456 aa, Homo sapiens
MTPILTVLICLGLSLGPRTHVQAGHLPKPTLWAEPGSVITQGSPVTLRCQGGQETQEYRLYREKKTALWITRIPQELVKKGQFPIPSITWEHAGRYRCYYGSDTAGRSESSDPLELVVTGAYIKPTLSAQPSPVVNSGGNVILQCDSQVAFDGFSLCKEGEDEHPQCLNSQPHARGSSRAIFSVGPVSPSRRWWYRCYAYDSNSPYEWSLPSDLLELLVLGVSKKPSLSVQPGPIVAPEETLTLQCGSDAGYNRFVLYKDGERDFLQLAGAQPQAGLSQANFTLGPVSRSYGGQYRCYGAHNLSSEWSAPSDPLDILIAGQFYDRVSLSVQPGPTVASGENVTLLCQSQGWMQTFLLTKEGAADDPWRLRSTYQSQKYQAEFPMGPVTSAHAGTYRCYGSQSSKPYLLTHPSDPLELVVSGPSGGPSSPTTGPTSTSAGPEDQPLTPTGSDPQSGE

SEQ ID NO: 390 - protein, 597 aa, Homo sapiens
MTPIVTVLICLGLSLGPRTRVQTGTIPKPTLWAEPDSVITQGSPVTLSCQGSLEAQEYRLYREKKSASWITRIRPELVKNGQFHIPSITWEHTGRYGCQYYSRARWSELSDPLVLVMTGAYPKPTLSAQPSPVVTSGGRVTLQCESQVAFGGFILCKEGEDEHPQCLNSQPHARGSSRAIFSVGPVSPNRRWSHRCYGYDLNSPYVWSSPSDLLELLVPGVSKKPSLSVQPGPVMAPGESLTLQCVSDVGYDRFVLYKEGERDLRQLPGRQPQAGLSQANFTLGPVSRSYGGQYRCYGAHNLSSECSAPSDPLDILITGQIRGTPFISVQPGPTVASGENVTLLCQSWRQFHTFLLTKAGAADAPLRLRSIHEYPKYQAEFPMSPVTSAHAGTYRCYGSLNSDPYLLSHPSEPLELVVSGPSMGSSPPPTGPISTPGPEDQPLTPTGSDPQSGLGRHLGVVIGILVAVVLLLLLLLLLFLILRHRRQGKHWTSTQRKADFQHPAGAVGPEPTDRGLQWRSSPAADAQEENLYAAVKDTQPEDGVEMDTRAAASEAPQDVTYAQLHSLTLRRKATEPPPSQEREPPAEPSIYATLAIH

SEQ ID NO: 391 - protein, 598 aa, Homo sapiens
MTPIVTVLICLGLSLGPRTRVQTGTIPKPTLWAEPDSVITQGSPVTLSCQGSLEAQEYRLYREKKSASWITRIRPELVKNGQFHIPSITWEHTGRYGCQYYSRARWSELSDPLVLVMTGAYPKPTLSAQPSPVVTSGGRVTLQCESQVAFGGFILCKEGEDEHPQCLNSQPHARGSSRAIFSVGPVSPNRRWSHRCYGYDLNSPYVWSSPSDLLELLVPGVSKKPSLSVQPGPVMAPGESLTLQCVSDVGYDRFVLYKEGERDLRQLPGRQPQAGLSQANFTLGPVSRSYGGQYRCYGAHNLSSECSAPSDPLDILITGQIRGTPFISVQPGPTVASGENVTLLCQSWRQFHTFLLTKAGAADAPLRLRSIHEYPKYQAEFPMSPVTSAHAGTYRCYGSLNSDPYLLSHPSEPLELVVSGPSMGSSPPPTGPISTPAGPEDQPLTPTGSDPQSGLGRHLGVVIGILVAVVLLLLLLLLLFLILRHRRQGKHWTSTQRKADFQHPAGAVGPEPTDRGLQWRSSPAADAQEENLYAAVKDTQPEDGVEMDTRAAASEAPQDVTYAQLHSLTLRRKATEPPPSQEREPPAEPSIYATLAIH

SEQ ID NO: 392 - protein, 510 aa, Homo sapiens
MTPIVTVLICLGLSLGPRTRVQTGTIPKPTLWAEPDSVITQGSPVTLSCQGSLEAQEYRLYREKKSASWITRIRPELVKNGQFHIPSITWEHTGRYGCQYYSRARWSELSDPLVLVMTGAYPKPTLSAQPSPVVTSGGRVTLQCESQVAFGGFILCKEGEDEHPQCLNSQPHARGSSRAIFSVGPVSPNRRWSHRCYGYDLNSPYVWSSPSDLLELLVPGVSKKPSLSVQPGPVMAPGESLTLQCVSDVGYDRFVLYKEGERDLRQLPGRQPQAGLSQANFTLGPVSRSYGGQYRCYGAHNLSSECSAPSDPLDILITGQIRGTPFISVQPGPTVASGENVTLLCQSWRQFHTFLLTKAGAADAPLRLRSIHEYPKYQAEFPMSPVTSAHAGTYRCYGSLNSDPYLLSHPSEPLELVVSGPSMGSSPPPTGPISTPAGPEDQPLTPTGSDPQSGLGRHLGVVIGILVAVVLLLLLLLLLFLILRHRRQGKHWTSSPAQLPTPRKKTSMLP

SEQ ID NO: 393 - protein, 482 aa, Homo sapiens
MTGAYPKPTLSAQPSPVVTSGGRVTLQCESQVAFGGFILCKEGEDEHPQCLNSQPHARGSSRAIFSVGPVSPNRRWSHRCYGYDLNSPYVWSSPSDLLELLVPGVSKKPSLSVQPGPVMAPGESLTLQCVSDVGYDRFVLYKEGERDLRQLPGRQPQAGLSQANFTLGPVSRSYGGQYRCYGAHNLSSECSAPSDPLDILITGQIRGTPFISVQPGPTVASGENVTLLCQSWRQFHTFLLTKAGAADAPLRLRSIHEYPKYQAEFPMSPVTSAHAGTYRCYGSLNSDPYLLSHPSEPLELVVSGPSMGSSPPPTGPISTPAGPEDQPLTPTGSDPQSGLGRHLGVVIGILVAVVLLLLLLLLLFLILRHRRQGKHWTSTQRKADFQHPAGAVGPEPTDRGLQWRSSPAADAQEENLYAAVKDTQPEDGVEMDTRAAASEAPQDVTYAQLHSLTLRRKATEPPPSQEREPPAEPSIYATLAIH

SEQ ID NO: 394 - protein, 489 aa, Homo sapiens
MTPIVTVLICLRLSLGPRTHVQAGTLPKPTLWAEPGSVITQGSPVTLWCQGILETQEYRLYREKKTAPWITRIPQEIVKKGQFPIPSITWEHTGRYRCFYGSHTAGWSEPSDPLELVVTGAYIKPTLSALPSPVVTSGGNVTLHCVSQVAFGSFILCKEGEDEHPQCLNSQPRTHGWSRAIFSVGPVSPSRRWSYRCYAYDSNSPHVWSLPSDLLELLVLGVSKKPSLSVQPGPIVAPGESLTLQCVSDVSYDRFVLYKEGERDFLQLPGPQPQAGLSQANFTLGPVSRSYGGQYRCSGAYNLSSEWSAPSDPLDILIAGQFRGRPFISVHPGPTVASGENVTLLCQSWGPFHTFLLTKAGAADAPLRLRSIHEYPKYQAEFPMSPVTSAHSGTYRCYGSLSSNPYLLSHPSDSLELMVSGAAETLSPPQNKSDSKAGAANTLSPSQNKTASHPQDYTVENLIRMGIAGLVLVVLGILLFEAQHSQRSL

SEQ ID NO: 395 - protein, 439 aa, Homo sapiens
MTPILTVLICLGLSLDPRTHVQAGPLPKPTLWAEPGSVITQGSPVTLRCQGSLETQEYHLYREKKTALWITRIPQELVKKGQFPILSITWEHAGRYCCIYGSHTAGLSESSDPLELVVTGAYSKPTLSALPSPVVTSGGNVTIQCDSQVAFDGFILCKEGEDEHPQCLNSHSHARGSSRAIFSVGPVSPSRRWSYRCYGYDSRAPYVWSLPSDLLGLLVPGVSKKPSLSVQPGPVVAPGEKLTFQCGSDAGYDRFVLYKEWGRDFLQRPGRQPQAGLSQANFTLGPVSRSYGGQYTCSGAYNLSSEWSAPSDPLDILITGQIRARPFLSVRPGPTVASGENVTLLCQSQGGMHTFLLTKEGAADSPLRLKSKRQSHKYQAEFPMSPVTSAHAGTYRCYGSLSSNPYLLTHPSDPLELVVSGAAETLSPPQNKSDSKAGE